European Patent Application EP 4 219 681 A1, published August 2, 2023. Title: Composition for diagnosis or treatment of inflammatory disease including microorganism. Applicant: ChunLab, Inc. The sequence listing filed with the application follows.

SEQUENCE LISTING (1 sequence)

SEQ ID NO: 1 - DNA, 1499 bp, Artificial Sequence
  Faecalibacterium cancerinhibens CLCC1 16S rRNA sequence
agagtttgatcctggctcaggacgaacgctggcggcgcgcctaacacatgcaagtcgaacgagcgagagagagcttgctttctcgagcgagtggcgaacgggtgagtaacgcgtgaggaacctgcctcaaagagggggacaacagttggaaacgactgctaataccgcataagcccacggctcggcatcgagcagagggaaaaggagcaatccgctttgagatggcctcgcgtccgattagctagttggtgaggtaatggcccaccaaggcgacgatcggtagccggactgagaggttgaacggccacattgggactgagacacggcccagactcctacgggaggcagcagtggggaatattgcacaatgggggaaaccctgatgcagcgacgccgcgtggaggaagaaggtcttcggattgtaaactcctgttgttggggaagataatgacggtacccaacaaggaagtgacggctaactacgtgccagcagccgcggtaaaacgtaggtcacaagcgttgtccggaattactgggtgtaaagggagcgcaggcgggaagacaagttggaagtgaaatctatgggctcaacccataaactgctttcaaaactgtttttcttgagtagtgcagaggtaggcggaattcccggtgtagcggtggaatgcgtagatatcgggaggaacaccagtggcgaaggcggcctactgggcaccaactgacgctgaggctcgaaagtgtgggtagcaaacaggattagataccctggtagtccacaccgtaaacgatgattactaggtgttggaggattgaccccttcagtgccgcagttaacacaataagtaatccacctggggagtacgaccgcaaggttgaaactcaaaggaattgacgggggcccgcacaagcagtggagtatgtggtttaattcgacgcaacgcgaagaaccttaccaagtcttgacatcccttgacagacatagaaatatgttttctcttcggagcaaggagacaggtggtgcatggttgtcgtcagctcgtgtcgtgagatgttgggttaagtcccgcaacgagcgcaacccttatggtcagttactacgcaagaggactctggccagactgccgttgacaaaacggaggaaggtggggatgacgtcaaatcatcatgccctttatgacttgggctacacacgtactacaatggcgttaaacaaagagaagcaagaccgcgaggtggagcaaaactcagaaacaacgtcccagttcggactgcaggctgcaactcgcctgcacgaagtcggaattgctagtaatcgtggatcagcatgccacggtgaatacgttcccgggccttgtacacaccgcccgtcacaccatgagagccggggggacccgaagtcggtagtctaaccgcaaggaggacgccgccgaaggtaaaactggtgattggggtgaagtcgtaacaaggtagccgtaggagaacctgcggctggatcacct